European Patent Application EP 4 293 127 A2, published December 20, 2023. Title: METHOD FOR REDUCING PRIMER DIMER FORMATION AND INCREASING AMPLIFICATION EFFICIENCY. Applicant: Seegene, Inc. The sequence listing filed with the application follows.

SEQUENCE LISTING (62 sequences)

SEQ ID NO: 1 - DNA, 24 bp, synthetic construct
  misc_feature 1..24: note = Synthetic oligonucleotide: UP-R1
  source 1..24: mol_type = other DNA
ggttctcaagcaacaatatcagct

SEQ ID NO: 2 - DNA, 11 bp, synthetic construct
  misc_feature 1..11: note = Synthetic oligonucleotide: UP-N-1
  source 1..11: mol_type = other DNA
agctgatattg

SEQ ID NO: 3 - DNA, 13 bp, synthetic construct
  misc_feature 1..13: note = Synthetic oligonucleotide: UP-N-2
  source 1..13: mol_type = other DNA
agctgatattgtt

SEQ ID NO: 4 - DNA, 15 bp, synthetic construct
  misc_feature 1..15: note = Synthetic oligonucleotide: UP-N-3
  source 1..15: mol_type = other DNA
agctgatattgttgc

SEQ ID NO: 5 - DNA, 22 bp, synthetic construct
  misc_feature 1..22: note = Synthetic oligonucleotide: UP-P-1
  source 1..22: mol_type = other DNA
ttggcttggcttggcttagctg

SEQ ID NO: 6 - DNA, 24 bp, synthetic construct
  misc_feature 1..24: note = Synthetic oligonucleotide: UP-P-2
  source 1..24: mol_type = other DNA
ttggcttggcttggcttagctgat

SEQ ID NO: 7 - DNA, 26 bp, synthetic construct
  misc_feature 1..26: note = Synthetic oligonucleotide: UP-P-3
  source 1..26: mol_type = other DNA
ttggcttggcttggcttagctgatat

SEQ ID NO: 8 - DNA, 21 bp, synthetic construct
  misc_feature 1..21: note = Synthetic oligonucleotide: UP-C-1
  source 1..21: mol_type = other DNA
ttggcttggcttggcttagct

SEQ ID NO: 9 - DNA, 22 bp, synthetic construct
  misc_feature 1..22: note = Synthetic oligonucleotide: UP-C-2
  source 1..22: mol_type = other DNA
ttggcttggcttggcttagctg

SEQ ID NO: 10 - DNA, 23 bp, synthetic construct
  misc_feature 1..23: note = Synthetic oligonucleotide: UP-C-3
  source 1..23: mol_type = other DNA
ttggcttggcttggcttagctga

SEQ ID NO: 11 - DNA, 24 bp, synthetic construct
  misc_feature 1..24: note = Synthetic oligonucleotide: UP-C-4
  source 1..24: mol_type = other DNA
ttggcttggcttggcttagctgat

SEQ ID NO: 12 - DNA, 21 bp, synthetic construct
  misc_feature 1..21: note = Synthetic oligonucleotide: NG-F4
  source 1..21: mol_type = other DNA
gcggacagttgtttttcgact

SEQ ID NO: 13 - DNA, 11 bp, synthetic construct
  misc_feature 1..11: note = Synthetic oligonucleotide: NG-N-1
  source 1..11: mol_type = other DNA
agtcgaaaaac

SEQ ID NO: 14 - DNA, 13 bp, synthetic construct
  misc_feature 1..13: note = Synthetic oligonucleotide: NG-N-2
  source 1..13: mol_type = other DNA
agtcgaaaaacaa

SEQ ID NO: 15 - DNA, 15 bp, synthetic construct
  misc_feature 1..15: note = Synthetic oligonucleotide: NG-N-3
  source 1..15: mol_type = other DNA
agtcgaaaaacaact

SEQ ID NO: 16 - DNA, 22 bp, synthetic construct
  misc_feature 1..22: note = Synthetic oligonucleotide: NG-P-1
  source 1..22: mol_type = other DNA
ttggcttggcttggcttagtcg

SEQ ID NO: 17 - DNA, 24 bp, synthetic construct
  misc_feature 1..24: note = Synthetic oligonucleotide: NG-P-2
  source 1..24: mol_type = other DNA
ttggcttggcttggcttagtcgaa

SEQ ID NO: 18 - DNA, 26 bp, synthetic construct
  misc_feature 1..26: note = Synthetic oligonucleotide: NG-P-3
  source 1..26: mol_type = other DNA
ttggcttggcttggcttagtcgaaaa

SEQ ID NO: 19 - DNA, 21 bp, synthetic construct
  misc_feature 1..21: note = Synthetic oligonucleotide: NG-C-1
  source 1..21: mol_type = other DNA
ttggcttggcttggcttagtc

SEQ ID NO: 20 - DNA, 22 bp, synthetic construct
  misc_feature 1..22: note = Synthetic oligonucleotide: NG-C-2
  source 1..22: mol_type = other DNA
ttggcttggcttggcttagtcg

SEQ ID NO: 21 - DNA, 23 bp, synthetic construct
  misc_feature 1..23: note = Synthetic oligonucleotide: NG-C-3
  source 1..23: mol_type = other DNA
ttggcttggcttggcttagtcga

SEQ ID NO: 22 - DNA, 24 bp, synthetic construct
  misc_feature 1..24: note = Synthetic oligonucleotide: NG-C-4
  source 1..24: mol_type = other DNA
ttggcttggcttggcttagtcgaa

SEQ ID NO: 23 - DNA, 24 bp, synthetic construct
  misc_feature 1..24: note = Synthetic oligonucleotide: UP-F1
  source 1..24: mol_type = other DNA
gcacaatttggatcattaaaaggt

SEQ ID NO: 24 - DNA, 20 bp, synthetic construct
  misc_feature 1..20: note = Synthetic oligonucleotide: NG-R2
  source 1..20: mol_type = other DNA
gtcgtatccgcatccgtcaa

SEQ ID NO: 25 - DNA, 25 bp, synthetic construct
  misc_feature 1..25: note = Synthetic oligonucleotide: UP-P1
  source 1..25: mol_type = other DNA
cccagctattgcacatggtgttgat

SEQ ID NO: 26 - DNA, 22 bp, synthetic construct
  misc_feature 1..22: note = Synthetic oligonucleotide: NG-P2
  source 1..22: mol_type = other DNA
tgtacggctccgttgtggcggt

SEQ ID NO: 27 - DNA, 24 bp, synthetic construct
  misc_feature 1..24: note = Synthetic oligonucleotide: UP-IR-2
  misc_feature 23: note = n is deoxyinosine
  source 1..24: mol_type = other DNA
ggttctcaagcaacaatatcagnt

SEQ ID NO: 28 - DNA, 24 bp, synthetic construct
  misc_feature 1..24: note = Synthetic oligonucleotide: UP-IR-3
  misc_feature 22: note = n is deoxyinosine
  source 1..24: mol_type = other DNA
ggttctcaagcaacaatatcanct

SEQ ID NO: 29 - DNA, 24 bp, synthetic construct
  misc_feature 1..24: note = Synthetic oligonucleotide: UP-IR-4
  misc_feature 21: note = n is deoxyinosine
  source 1..24: mol_type = other DNA
ggttctcaagcaacaatatcngct

SEQ ID NO: 30 - DNA, 24 bp, synthetic construct
  misc_feature 1..24: note = Synthetic oligonucleotide: UP-IR-5
  misc_feature 20: note = n is deoxyinosine
  source 1..24: mol_type = other DNA
ggttctcaagcaacaatatnagct

SEQ ID NO: 31 - DNA, 24 bp, synthetic construct
  misc_feature 1..24: note = Synthetic oligonucleotide: UP-IR-6
  misc_feature 19: note = n is deoxyinosine
  source 1..24: mol_type = other DNA
ggttctcaagcaacaatancagct

SEQ ID NO: 32 - DNA, 24 bp, synthetic construct
  misc_feature 1..24: note = Synthetic oligonucleotide: UP-IR-7
  misc_feature 18: note = n is deoxyinosine
  source 1..24: mol_type = other DNA
ggttctcaagcaacaatntcagct

SEQ ID NO: 33 - DNA, 24 bp, synthetic construct
  misc_feature 1..24: note = Synthetic oligonucleotide: UP-IR-8
  misc_feature 17: note = n is deoxyinosine
  source 1..24: mol_type = other DNA
ggttctcaagcaacaanatcagct

SEQ ID NO: 34 - DNA, 21 bp, synthetic construct
  misc_feature 1..21: note = Synthetic oligonucleotide: NG-IF-2
  misc_feature 20: note = n is deoxyinosine
  source 1..21: mol_type = other DNA
gcggacagttgtttttcgant

SEQ ID NO: 35 - DNA, 21 bp, synthetic construct
  misc_feature 1..21: note = Synthetic oligonucleotide: NG-IF-3
  misc_feature 19: note = n is deoxyinosine
  source 1..21: mol_type = other DNA
gcggacagttgtttttcgnct

SEQ ID NO: 36 - DNA, 21 bp, synthetic construct
  misc_feature 1..21: note = Synthetic oligonucleotide: NG-IF-4
  misc_feature 18: note = n is deoxyinosine
  source 1..21: mol_type = other DNA
gcggacagttgtttttcnact

SEQ ID NO: 37 - DNA, 21 bp, synthetic construct
  misc_feature 1..21: note = Synthetic oligonucleotide: NG-IF-5
  misc_feature 17: note = n is deoxyinosine
  source 1..21: mol_type = other DNA
gcggacagttgtttttngact

SEQ ID NO: 38 - DNA, 21 bp, synthetic construct
  misc_feature 1..21: note = Synthetic oligonucleotide: NG-IF-6
  misc_feature 16: note = n is deoxyinosine
  source 1..21: mol_type = other DNA
gcggacagttgttttncgact

SEQ ID NO: 39 - DNA, 21 bp, synthetic construct
  misc_feature 1..21: note = Synthetic oligonucleotide: NG-IF-7
  misc_feature 15: note = n is deoxyinosine
  source 1..21: mol_type = other DNA
gcggacagttgtttntcgact

SEQ ID NO: 40 - DNA, 21 bp, synthetic construct
  misc_feature 1..21: note = Synthetic oligonucleotide: NG-IF-8
  misc_feature 14: note = n is deoxyinosine
  source 1..21: mol_type = other DNA
gcggacagttgttnttcgact

SEQ ID NO: 41 - DNA, 28 bp, synthetic construct
  misc_feature 1..28: note = Synthetic oligonucleotide: UU-F1
  source 1..28: mol_type = other DNA
gcatatgatgaagcacacaacaaaatgg

SEQ ID NO: 42 - DNA, 22 bp, synthetic construct
  misc_feature 1..22: note = Synthetic oligonucleotide: UU-R1
  source 1..22: mol_type = other DNA
gctttggctgatgattgcgtag

SEQ ID NO: 43 - DNA, 22 bp, synthetic construct
  misc_feature 1..22: note = Synthetic oligonucleotide: MG-F1
  source 1..22: mol_type = other DNA
aaaacccacggaaatgatgaga

SEQ ID NO: 44 - DNA, 26 bp, synthetic construct
  misc_feature 1..26: note = Synthetic oligonucleotide: MG-R1
  source 1..26: mol_type = other DNA
ctcgttaatttacctattccattttg

SEQ ID NO: 45 - DNA, 20 bp, synthetic construct
  misc_feature 1..20: note = Synthetic oligonucleotide: NG-F1
  source 1..20: mol_type = other DNA
tacgcctgctactttcacgc

SEQ ID NO: 46 - DNA, 21 bp, synthetic construct
  misc_feature 1..21: note = Synthetic oligonucleotide: NG-R1
  source 1..21: mol_type = other DNA
caatggatcggtatcactcgc

SEQ ID NO: 47 - DNA, 27 bp, synthetic construct
  misc_feature 1..27: note = Synthetic oligonucleotide: CT-F1
  source 1..27: mol_type = other DNA
ttattcatccgaatggataaagcgtga

SEQ ID NO: 48 - DNA, 22 bp, synthetic construct
  misc_feature 1..22: note = Synthetic oligonucleotide: CT-R1
  source 1..22: mol_type = other DNA
aacaatgaatcctgagcaaagg

SEQ ID NO: 49 - DNA, 28 bp, synthetic construct
  misc_feature 1..28: note = Synthetic oligonucleotide: UU-F2
  misc_feature 26: note = n is deoxyinosine
  source 1..28: mol_type = other DNA
gcatatgatgaagcacacaacaaaangg

SEQ ID NO: 50 - DNA, 22 bp, synthetic construct
  misc_feature 1..22: note = Synthetic oligonucleotide: MG-F2
  misc_feature 18: note = n is deoxyinosine
  source 1..22: mol_type = other DNA
aaaacccacggaaatgangaga

SEQ ID NO: 51 - DNA, 20 bp, synthetic construct
  misc_feature 1..20: note = Synthetic oligonucleotide: NG-F2
  misc_feature 17: note = n is deoxyinosine
  source 1..20: mol_type = other DNA
tacgcctgctactttcncgc

SEQ ID NO: 52 - DNA, 27 bp, synthetic construct
  misc_feature 1..27: note = Synthetic oligonucleotide: CT-F2
  misc_feature 25: note = n is deoxyinosine
  source 1..27: mol_type = other DNA
ttattcatccgaatggataaagcgnga

SEQ ID NO: 53 - DNA, 28 bp, synthetic construct
  misc_feature 1..28: note = Synthetic oligonucleotide: UU-F3
  misc_feature 13: note = n is deoxyinosine
  misc_feature 26: note = n is deoxyinosine
  source 1..28: mol_type = other DNA
gcatatgatgaancacacaacaaaangg

SEQ ID NO: 54 - DNA, 22 bp, synthetic construct
  misc_feature 1..22: note = Synthetic oligonucleotide: MG-F3
  misc_feature 10: note = n is deoxyinosine
  misc_feature 18: note = n is deoxyinosine
  source 1..22: mol_type = other DNA
aaaacccacngaaatgangaga

SEQ ID NO: 55 - DNA, 20 bp, synthetic construct
  misc_feature 1..20: note = Synthetic oligonucleotide: NG-F3
  misc_feature 10: note = n is deoxyinosine
  misc_feature 17: note = n is deoxyinosine
  source 1..20: mol_type = other DNA
tacgcctgcnactttcncgc

SEQ ID NO: 56 - DNA, 27 bp, synthetic construct
  misc_feature 1..27: note = Synthetic oligonucleotide: CT-F3
  misc_feature 14: note = n is deoxyinosine
  misc_feature 25: note = n is deoxyinosine
  source 1..27: mol_type = other DNA
ttattcatccgaanggataaagcgnga

SEQ ID NO: 57 - DNA, 27 bp, synthetic construct
  misc_feature 1..27: note = UU-P1
  source 1..27: mol_type = other DNA
cacttcaccagatacataacccccgcc

SEQ ID NO: 58 - DNA, 28 bp, synthetic construct
  misc_feature 1..28: note = MG-P1
  source 1..28: mol_type = other DNA
acacctcttgctgttcttgaaagaactc

SEQ ID NO: 59 - DNA, 22 bp, synthetic construct
  misc_feature 1..22: note = NG-P1
  source 1..22: mol_type = other DNA
tgcccctcattggcgtgtttcg

SEQ ID NO: 60 - DNA, 29 bp, synthetic construct
  misc_feature 1..29: note = CT-P1
  source 1..29: mol_type = other DNA
cattgtaaagatatggtctgcttcgaccg

SEQ ID NO: 61 - skipped

SEQ ID NO: 62 - DNA, 26 bp, synthetic construct
  misc_feature 1..26: note = primer
  source 1..26: mol_type = other DNA
aaaaaaaaaaaaaaaaaaaaggggaa